European Patent Application EP 4 512 427 A1, published February 26, 2025. Title: ANTIBODY-DRUG CONJUGATES BASED ON MOLECULAR GLUE DEGRADERS AND USES THEREOF. Applicant: MABLINK BIOSCIENCE. Application EP. The sequence listing filed with the application follows.

SEQUENCE LISTING (8 sequences)

SEQ ID NO: 1 - protein, 449 aa, synthetic construct
EVQLVESGGGVVQPGRSLRLSCSASGFTFSGYGLSWVRQAPGKGLEWVAMISSGGSYTYYADSVKGRFAISRDNAKNTLFLQMDSLRPEDTGVYFCARHGDDPAWFAYWGQGTPVTVSSASTKGPSVFPLAPSSKSTSGGTAALGCLVKDYFPEPVTVSWNSGALTSGVHTFPAVLQSSGLYSLSSVVTVPSSSLGTQTYICNVNHKPSNTKVDKKVEPKSCDKTHTCPPCPAPEAAGGPSVFLFPPKPKDTLMISRTPEVTCVVVDVSHEDPEVKFNWYVDGVEVHNAKTKPREEQYNSTYRVVSVLTVLHQDWLNGKEYKCKVSNKALPAPIEKTISKAKGQPREPQVYTLPPSRDELTKNQVSLTCLVKGFYPSDIAVEWESNGQPENNYKTTPPVLDSDGSFFLYSKLTVDKSRWQQGNVFSCSVMHEALHNHYTQKSLSLSPGK

SEQ ID NO: 2 - protein, 217 aa, synthetic construct
DIQLTQSPSSLSASVGDRVTITCSVSSSISSNNLHWYQQKPGKAPKPWIYGTSNLASGVPSRFSGSGSGTDYTFTISSLQPEDIATYYCQQWSSYPYMYTFGQGTKVEIKRTVAAPSVFIFPPSDEQLKSGTASVVCLLNNFYPREAKVQWKVDNALQSGNSQESVTEQDSKDSTYSLSSTLTLSKADYEKHKVYACEVTHQGLSSPVTKSFNRGEC

SEQ ID NO: 3 - protein, 450 aa, synthetic construct
QVQLQQSGSELKKPGASVKVSCKASGYTFTNYGVNWIKQAPGQGLQWMGWINPNTGEPTFDDDFKGRFAFSLDTSVSTAYLQISSLKADDTAVYFCSRSRGKNEAWFAYWGQGTLVTVSSASTKGPSVFPLAPSSKSTSGGTAALGCLVKDYFPEPVTVSWNSGALTSGVHTFPAVLQSSGLYSLSSVVTVPSSSLGTQTYICNVNHKPSNTKVDKRVEPKSCDKTHTCPPCPAPELLGGPSVFLFPPKPKDTLMISRTPEVTCVVVDVSHEDPEVKFNWYVDGVEVHNAKTKPREEQYNSTYRVVSVLTVLHQDWLNGKEYKCKVSNKALPAPIEKTISKAKGQPREPQVYTLPPSREEMTKNQVSLTCLVKGFYPSDIAVEWESNGQPENNYKTTPPVLDSDGSFFLYSKLTVDKSRWQQGNVFSCSVMHEALHNHYTQKSLSLSPGK

SEQ ID NO: 4 - protein, 219 aa, synthetic construct
DIQLTQSPLSLPVTLGQPASISCRSSQSLVHRNGNTYLHWFQQRPGQSPRLLIYTVSNRFSGVPDRFSGSGSGTDFTLKISRVEAEDVGVYFCSQSSHVPPTFGAGTRLEIKRTVAAPSVFIFPPSDEQLKSGTASVVCLLNNFYPREAKVQWKVDNALQSGNSQESVTEQDSKDSTYSLSSTLTLSKADYEKHKVYACEVTHQGLSSPVTKSFNRGEC

SEQ ID NO: 5 - protein, 448 aa, synthetic construct
QVQLQQPGAEVVKPGASVKMSCKASGYTFTSYYIHWIKQTPGQGLEWVGVIYPGNDDISYNQKFQGKATLTADKSSTTAYMQLSSLTSEDSAVYYCAREVRLRYFDVWGQGTTVTVSSASTKGPSVFPLAPSSKSTSGGTAALGCLVKDYFPEPVTVSWNSGALTSGVHTFPAVLQSSGLYSLSSVVTVPSSSLGTQTYICNVNHKPSNTKVDKKVEPKSCDKTHTCPPCPAPELLGGPSVFLFPPKPKDTLMISRTPEVTCVVVDVSHEDPEVKFNWYVDGVEVHNAKTKPREEQYNSTYRVVSVLTVLHQDWLNGKEYKCKVSNKALPAPIEKTISKAKGQPREPQVYTLPPSRDELTKNQVSLTCLVKGFYPSDIAVEWESNGQPENNYKTTPPVLDSDGSFFLYSKLTVDKSRWQQGNVFSCSVMHEALHNHYTQKSLSLSPGK

SEQ ID NO: 6 - protein, 219 aa, synthetic construct
EIVLTQSPGSLAVSPGERVTMSCKSSQSVFFSSSQKNYLAWYQQIPGQSPRLLIYWASTRESGVPDRFTGSGSGTDFTLTISSVQPEDLAIYYCHQYLSSRTFGQGTKLEIKRTVAAPSVFIFPPSDEQLKSGTASVVCLLNNFYPREAKVQWKVDNALQSGNSQESVTEQDSKDSTYSLSSTLTLSKADYEKHKVYACEVTHQGLSSPVTKSFNRGEC

SEQ ID NO: 7 - protein, 446 aa, synthetic construct
QIQLQQSGPEVVKPGASVKISCKASGYTFTDYYITWVKQKPGQGLEWIGWIYPGSGNTKYNEKFKGKATLTVDTSSSTAFMQLSSLTSEDTAVYFCANYGNYWFAYWGQGTQVTVSAASTKGPSVFPLAPSSKSTSGGTAALGCLVKDYFPEPVTVSWNSGALTSGVHTFPAVLQSSGLYSLSSVVTVPSSSLGTQTYICNVNHKPSNTKVDKKVEPKSCDKTHTCPPCPAPEAAGGPSVFLFPPKPKDTLMISRTPEVTCVVVDVSHEDPEVKFNWYVDGVEVHNAKTKPREEQYNSTYRVVSVLTVLHQDWLNGKEYKCKVSNKALPAPIEKTISKAKGQPREPQVYTLPPSRDELTKNQVSLTCLVKGFYPSDIAVEWESNGQPENNYKTTPPVLDSDGSFFLYSKLTVDKSRWQQGNVFSCSVMHEALHNHYTQKSLSLSPG

SEQ ID NO: 8 - protein, 218 aa, synthetic construct
DIVLTQSPASLAVSLGQRATISCKASQSVDFDGDSYMNWYQQKPGQPPKVLIYAASNLESGIPARFSGSGSGTDFTLNIHPVEEEDAATYYCQQSNEDPWTFGGGTKLEIKRTVAAPSVFIFPPSDEQLKSGTASVVCLLNNFYPREAKVQWKVDNALQSGNSQESVTEQDSKDSTYSLSSTLTLSKADYEKHKVYACEVTHQGLSSPVTKSFNRGEC